European Patent Specification EP 3 922 645 B1, published May 14, 2025. Title: ANTI-PRO/LATENT-MYOSTATIN ANTIBODIES AND USES THEREOF. Applicant: Scholar Rock, Inc. Application Not Yet Assigned. The sequence listing filed with the application follows.

SEQUENCE LISTING (65 sequences)

SEQ ID NO: 1 - protein, 6 aa, Artificial Sequence
  Synthetic Polypeptide
SSYGMH

SEQ ID NO: 2 - protein, 10 aa, Artificial Sequence
  Synthetic Polypeptide
GFTFSSYGMH

SEQ ID NO: 3 - protein, 10 aa, Artificial Sequence
  Synthetic Polypeptide
GFAFSSYGMH

SEQ ID NO: 4 - protein, 17 aa, Artificial Sequence
  Synthetic Polypeptide
VISYDGSNKYYADSVKG

SEQ ID NO: 5 - protein, 7 aa, Artificial Sequence
  Synthetic Polypeptide
ISYDGSN

SEQ ID NO: 6 - protein, 17 aa, Artificial Sequence
  Synthetic Polypeptide
VISYDGSIKYYADSVKG

SEQ ID NO: 7 - protein, 7 aa, Artificial Sequence
  Synthetic Polypeptide
ISYDGSI

SEQ ID NO: 8 - protein, 17 aa, Artificial Sequence
  Synthetic Polypeptide
VISYDGNNKYYADSVKG

SEQ ID NO: 9 - protein, 7 aa, Artificial Sequence
  Synthetic Polypeptide
ISYDGNN

SEQ ID NO: 10 - protein, 17 aa, Artificial Sequence
  Synthetic Polypeptide
DLLVRFLEWSHYYGMDV

SEQ ID NO: 11 - protein, 17 aa, Artificial Sequence
  Synthetic Polypeptide
DLLVRFLEWSHKYGMDV

SEQ ID NO: 12 - protein, 13 aa, Artificial Sequence
  Synthetic Polypeptide
SGSSSNIGSNTVH

SEQ ID NO: 13 - protein, 8 aa, Artificial Sequence
  Synthetic Polypeptide
SSNIGSNT

SEQ ID NO: 14 - protein, 13 aa, Artificial Sequence
  Synthetic Polypeptide
SGSTSNIGSNTVH

SEQ ID NO: 15 - protein, 8 aa, Artificial Sequence
  Synthetic Polypeptide
TSNIGSNT

SEQ ID NO: 16 - protein, 13 aa, Artificial Sequence
  Synthetic Polypeptide
SGSSSNIGGNTVH

SEQ ID NO: 17 - protein, 8 aa, Artificial Sequence
  Synthetic Polypeptide
SSNIGGNT

SEQ ID NO: 18 - protein, 7 aa, Artificial Sequence
  Synthetic Polypeptide
SDNQRPS

SEQ ID NO: 19 - protein, 3 aa, Artificial Sequence
  Synthetic Polypeptide
SDN

SEQ ID NO: 20 - protein, 7 aa, Artificial Sequence
  Synthetic Polypeptide
SDDQRPS

SEQ ID NO: 21 - protein, 3 aa, Artificial Sequence
  Synthetic Polypeptide
SDD

SEQ ID NO: 22 - protein, 10 aa, Artificial Sequence
  Synthetic Polypeptide
AAWDDSLNGV

SEQ ID NO: 23 - protein, 10 aa, Artificial Sequence
  Synthetic Polypeptide
AAWDESLNGV

SEQ ID NO: 24 - protein, 126 aa, Artificial Sequence
  Synthetic Polypeptide
QIQLVQSGGGVVQPGRSLRLSCAASGFTFSSYGMHWVRQAPGKGLEWVAVISYDGSNKYYADSVKGRFTISRDNSKNTLYLQMNSLRAEDTAVYYCARDLLVRFLEWSHYYGMDVWGQGTTVTVSS

SEQ ID NO: 25 - protein, 126 aa, Artificial Sequence
  Synthetic Polypeptide
QVQLVESGGGVVQPGRSLRLSCAASGFTFSSYGMHWVRQAPGKGLEWVAVISYDGSNKYYADSVKGRFTISRDNSKNTLYLQMNSLRAEDTAVYYCARDLLVRFLEWSHYYGMDVWGQGTTVTVSS

SEQ ID NO: 26 - protein, 126 aa, Artificial Sequence
  Synthetic Polypeptide
QIQLVQSGGGVVQPGRSLRLSCAASGFAFSSYGMHWVRQAPGKGLEWVAVISYDGSIKYYADSVKGRFTISRDNSKNTLYLQMNSLRAEDTAVYYCARDLLVRFLEWSHKYGMDVWGQGTTVTVSS

SEQ ID NO: 27 - protein, 126 aa, Artificial Sequence
  Synthetic Polypeptide
QVQLVESGGGVVQPGRSLRLSCAASGFAFSSYGMHWVRQAPGKGLEWVAVISYDGSIKYYADSVKGRFTISRDNSKNTLYLQMNSLRAEDTAVYYCARDLLVRFLEWSHKYGMDVWGQGTTVTVSS

SEQ ID NO: 28 - protein, 126 aa, Artificial Sequence
  Synthetic Polypeptide
QIQLVQSGGGVVQPGRSLRLSCAASGFAFSSYGMHWVRQAPGKGLEWVAVISYDGNNKYYADSVKGRFTISRDNSKNTLYLQMNSLRAEDTAVYYCARDLLVRFLEWSHKYGMDVWGQGTTVTVSS

SEQ ID NO: 29 - protein, 126 aa, Artificial Sequence
  Synthetic Polypeptide
QVQLVESGGGVVQPGRSLRLSCAASGFAFSSYGMHWVRQAPGKGLEWVAVISYDGNNKYYADSVKGRFTISRDNSKNTLYLQMNSLRAEDTAVYYCARDLLVRFLEWSHKYGMDVWGQGTTVTVSS

SEQ ID NO: 30 - protein, 109 aa, Artificial Sequence
  Synthetic Polypeptide
QPVLTQPPSASGTPGQRVTISCSGSSSNIGSNTVHWYQQLPGTAPKLLIYSDNQRPSGVPDRFSGSKSGTSASLVISGLQSDDEADYYCAAWDDSLNGVFGGGTKLTVL

SEQ ID NO: 31 - protein, 109 aa, Artificial Sequence
  Synthetic Polypeptide
QSVLTQPPSASGTPGQRVTISCSGSSSNIGSNTVHWYQQLPGTAPKLLIYSDNQRPSGVPDRFSGSKSGTSASLAISGLQSEDEADYYCAAWDDSLNGVFGGGTKLTVL

SEQ ID NO: 32 - protein, 109 aa, Artificial Sequence
  Synthetic Polypeptide
QPVLTQPPSASGTPGQRVTISCSGSTSNIGSNTVHWYQQLPGTAPKLLIYSDDQRPSGVPDRFSGSKSGTSASLVISGLQSDDEADYYCAAWDESLNGVFGGGTKLTVL

SEQ ID NO: 33 - protein, 109 aa, Artificial Sequence
  Synthetic Polypeptide
QSVLTQPPSASGTPGQRVTISCSGSTSNIGSNTVHWYQQLPGTAPKLLIYSDDQRPSGVPDRFSGSKSGTSASLAISGLQSEDEADYYCAAWDESLNGVFGGGTKLTVL

SEQ ID NO: 34 - protein, 109 aa, Artificial Sequence
  Synthetic Polypeptide
QPVLTQPPSASGTPGQRVTISCSGSSSNIGGNTVHWYQQLPGTAPKLLIYSDDQRPSGVPDRFSGSKSGTSASLVISGLQSDDEADYYCAAWDESLNGVFGGGTKLTVL

SEQ ID NO: 35 - protein, 109 aa, Artificial Sequence
  Synthetic Polypeptide
QSVLTQPPSASGTPGQRVTISCSGSSSNIGGNTVHWYQQLPGTAPKLLIYSDDQRPSGVPDRFSGSKSGTSASLAISGLQSEDEADYYCAAWDESLNGVFGGGTKLTVL

SEQ ID NO: 36 - protein, 98 aa, Artificial Sequence
  Synthetic Polypeptide
QVQLVESGGGVVQPGRSLRLSCAASGFTFSSYGMHWVRQAPGKGLEWVAVISYDGSNKYYADSVKGRFTISRDNSKNTLYLQMNSLRAEDTAVYYCAR

SEQ ID NO: 37 - protein, 98 aa, Artificial Sequence
  Synthetic Polypeptide
QSVLTQPPSASGTPGQRVTISCSGSSSNIGSNTVNWYQQLPGTAPKLLIYSNNQRPSGVPDRFSGSKSGTSASLAISGLQSEDEADYYCAAWDDSLNG

SEQ ID NO: 38 - DNA, 378 bp, Artificial Sequence
  Synthetic Polynucleotide
cagatccagctggtgcagtctgggggaggcgtggtccagcctgggaggtccctgagactctcctgtgcagcgtctggattcaccttcagtagctatggcatgcactgggtccgccaggctccaggcaaggggctggagtgggtggcagttatatcatatgatggaagtaataaatactatgcagactccgtgaagggccgattcaccatctccagagacaattccaagaacacgctgtatctgcaaatgaacagcctgagagccgaggacacggctgtgtattactgtgcgagagatctcctggtgcgatttttggagtggtcgcactactacggtatggacgtctggggccaagggaccacggtcaccgtctcctca

SEQ ID NO: 39 - DNA, 378 bp, Artificial Sequence
  Synthetic Polynucleotide
caggtgcagctggtggagtctgggggaggcgtggtccagcctgggaggtccctgagactctcctgtgcagcgtctggattcaccttcagtagctatggcatgcactgggtccgccaggctccaggcaaggggctggagtgggtggcagttatatcatatgatggaagtaataaatactatgcagactccgtgaagggccgattcaccatctccagagacaattccaagaacacgctgtatctgcaaatgaacagcctgagagccgaggacacggctgtgtattactgtgcgagagatctcctggtgcgatttttggagtggtcgcactactacggtatggacgtctggggccaagggaccacggtcaccgtctcctca

SEQ ID NO: 40 - DNA, 378 bp, Artificial Sequence
  Synthetic Polynucleotide
cagatccagctggtgcagtctgggggaggcgtggtccagcctgggaggtccctgagactctcctgtgcagcgtctggattcgccttcagtagctatggcatgcactgggtccgccaggctccaggcaaggggctggagtgggtggcagttatatcatatgatggaagtatcaaatactatgcagactccgtgaagggccgattcaccatctccagagacaattccaagaacacgctgtatctgcaaatgaacagcctgagagccgaggacacggctgtgtattactgtgcgagagatctcctggtgcgatttttggagtggtcgcacaagtacggtatggacgtctggggccaagggaccacggtcaccgtctcctca

SEQ ID NO: 41 - DNA, 378 bp, Artificial Sequence
  Synthetic Polynucleotide
caggtgcagctggtggagtctgggggaggcgtggtccagcctgggaggtccctgagactctcctgtgcagcgtctggattcgccttcagtagctatggcatgcactgggtccgccaggctccaggcaaggggctggagtgggtggcagttatatcatatgatggaagtatcaaatactatgcagactccgtgaagggccgattcaccatctccagagacaattccaagaacacgctgtatctgcaaatgaacagcctgagagccgaggacacggctgtgtattactgtgcgagagatctcctggtgcgatttttggagtggtcgcacaagtacggtatggacgtctggggccaagggaccacggtcaccgtctcctca

SEQ ID NO: 42 - DNA, 378 bp, Artificial Sequence
  Synthetic Polynucleotide
cagatccagctggtgcagtctgggggaggcgtggtccagcctgggaggtccctgagactctcctgtgcagcgtctggattcgccttcagtagctatggcatgcactgggtccgccaggctccaggcaaggggctggagtgggtggcagttatatcatatgatggaaataataaatactatgcagactccgtgaagggccgattcaccatctccagagacaattccaagaacacgctgtatctgcaaatgaacagcctgagagccgaggacacggctgtgtattactgtgcgagagatctcctggtgcgatttttggagtggtcgcacaagtacggtatggacgtctggggccaagggaccacggtcaccgtctcctca

SEQ ID NO: 43 - DNA, 378 bp, Artificial Sequence
  Synthetic Polynucleotide
caggtgcagctggtggagtctgggggaggcgtggtccagcctgggaggtccctgagactctcctgtgcagcgtctggattcgccttcagtagctatggcatgcactgggtccgccaggctccaggcaaggggctggagtgggtggcagttatatcatatgatggaaataataaatactatgcagactccgtgaagggccgattcaccatctccagagacaattccaagaacacgctgtatctgcaaatgaacagcctgagagccgaggacacggctgtgtattactgtgcgagagatctcctggtgcgatttttggagtggtcgcacaagtacggtatggacgtctggggccaagggaccacggtcaccgtctcctca

SEQ ID NO: 44 - DNA, 327 bp, Artificial Sequence
  Synthetic Polynucleotide
cagcctgtgctgactcagccaccctcagcgtctgggacccccgggcagagggtcaccatctcttgttctggaagcagctccaacatcggaagtaatactgtccactggtaccagcaactcccaggaacggcccccaaactcctcatctatagtgataatcagcgcccctcaggggtccctgaccgattctctggctccaagtctggcacctcagcctccctggtcatcagtgggctccagtctgacgatgaggctgattattactgtgcagcatgggatgacagcctgaatggggtgttcggcggagggaccaagctgaccgtccta

SEQ ID NO: 45 - DNA, 327 bp, Artificial Sequence
  Synthetic Polynucleotide
cagtctgtgctgactcagccaccctcagcgtctgggacccccgggcagagggtcaccatctcttgttctggaagcagctccaacatcggaagtaatactgtccactggtaccagcaactcccaggaacggcccccaaactcctcatctatagtgataatcagcgcccctcaggggtccctgaccgattctctggctccaagtctggcacctcagcctccctggccatcagtgggctccagtctgaggatgaggctgattattactgtgcagcatgggatgacagcctgaatggggtgttcggcggagggaccaagctgaccgtccta

SEQ ID NO: 46 - DNA, 327 bp, Artificial Sequence
  Synthetic Polynucleotide
cagcctgtgctgactcagccaccctcagcgtctgggacccccgggcagagggtcaccatctcttgttctggaagcacctccaacatcggaagtaatactgtccactggtaccagcaactcccaggaacggcccccaaactcctcatctatagtgatgatcagcgcccctcaggggtccctgaccgattctctggctccaagtctggcacctcagcctccctggtcatcagtgggctccagtctgacgatgaggctgattattactgtgcagcatgggatgagagcctgaatggggtgttcggcggagggaccaagctgaccgtccta

SEQ ID NO: 47 - DNA, 327 bp, Artificial Sequence
  Synthetic Polynucleotide
cagtctgtgctgactcagccaccctcagcgtctgggacccccgggcagagggtcaccatctcttgttctggaagcacctccaacatcggaagtaatactgtccactggtaccagcaactcccaggaacggcccccaaactcctcatctatagtgatgatcagcgcccctcaggggtccctgaccgattctctggctccaagtctggcacctcagcctccctggccatcagtgggctccagtctgaggatgaggctgattattactgtgcagcatgggatgagagcctgaatggggtgttcggcggagggaccaagctgaccgtccta

SEQ ID NO: 48 - DNA, 327 bp, Artificial Sequence
  Synthetic Polynucleotide
cagcctgtgctgactcagccaccctcagcgtctgggacccccgggcagagggtcaccatctcttgttctggaagcagctccaacatcggaggaaatactgtccactggtaccagcaactcccaggaacggcccccaaactcctcatctatagtgatgatcagcgcccctcaggggtccctgaccgattctctggctccaagtctggcacctcagcctccctggtcatcagtgggctccagtctgacgatgaggctgattattactgtgcagcatgggatgagagcctgaatggggtgttcggcggagggaccaagctgaccgtccta

SEQ ID NO: 49 - DNA, 327 bp, Artificial Sequence
  Synthetic Polynucleotide
cagtctgtgctgactcagccaccctcagcgtctgggacccccgggcagagggtcaccatctcttgttctggaagcagctccaacatcggaggaaatactgtccactggtaccagcaactcccaggaacggcccccaaactcctcatctatagtgatgatcagcgcccctcaggggtccctgaccgattctctggctccaagtctggcacctcagcctccctggccatcagtgggctccagtctgaggatgaggctgattattactgtgcagcatgggatgagagcctgaatggggtgttcggcggagggaccaagctgaccgtccta

SEQ ID NO: 50 - protein, 452 aa, Artificial Sequence
  Synthetic Polypeptide
QVQLVESGGGVVQPGRSLRLSCAASGFTFSSYGMHWVRQAPGKGLEWVAVISYDGSNKYYADSVKGRFTISRDNSKNTLYLQMNSLRAEDTAVYYCARDLLVRFLEWSHYYGMDVWGQGTTVTVSSASTKGPSVFPLAPCSRSTSESTAALGCLVKDYFPEPVTVSWNSGALTSGVHTFPAVLQSSGLYSLSSVVTVPSSSLGTKTYTCNVDHKPSNTKVDKRVESKYGPPCPPCPAPEFLGGPSVFLFPPKPKDTLMISRTPEVTCVVVDVSQEDPEVQFNWYVDGVEVHNAKTKPREEQFNSTYRVVSVLTVLHQDWLNGKEYKCKVSNKGLPSSIEKTISKAKGQPREPQVYTLPPSQEEMTKNQVSLTCLVKGFYPSDIAVEWESNGQPENNYKTTPPVLDSDGSFFLYSRLTVDKSRWQEGNVFSCSVMHEALHNHYTQKSLSLSLG

SEQ ID NO: 51 - protein, 215 aa, Artificial Sequence
  Synthetic Polypeptide
QSVLTQPPSASGTPGQRVTISCSGSSSNIGSNTVHWYQQLPGTAPKLLIYSDNQRPSGVPDRFSGSKSGTSASLAISGLQSEDEADYYCAAWDDSLNGVFGGGTKLTVLGQPKAAPSVTLFPPSSEELQANKATLVCLISDFYPGAVTVAWKADSSPVKAGVETTTPSKQSNNKYAASSYLSLTPEQWKSHRSYSCQVTHEGSTVEKTVAPTECS

SEQ ID NO: 52 - protein, 352 aa, Homo sapiens [sequence omitted]

SEQ ID NO: 53 - protein, 352 aa, Rattus rattus
NEDSEREANVEKEGLCNACAWRQNTRYSRIEAIKIQILSKLRLETAPNISKDAIRQLLPRAPPLRELIDQYDVQRDDSSDGSLEDDDYHATTETIITMPTESDFLMQADGKPKCCFFKFSSKIQYNKVVKAQLWIYLRAVKTPTTVFVQILRLIKPMKDGTRYTGIRSLKLDMSPGTGIWQSIDVKTVLQNWLKQPESNLGIEIKALDENGHDLAVTFPGPGEDGLNPFLEVKVTDTPKRSRRDFGLDCDEHSTESRCCRYPLTVDFEAFGWDWIIAPKRYKANYCSGECEFVFLQKYPHTHLVHQANPRGSAGPCCTPTKMSPINMLYFNGKEQIIYGKIPAMVVDRCGCS

SEQ ID NO: 54 - protein, 352 aa, Mus musculus
NEGSEREENVEKEGLCNACAWRQNTRYSRIEAIKIQILSKLRLETAPNISKDAIRQLLPRAPPLRELIDQYDVQRDDSSDGSLEDDDYHATTETIITMPTESDFLMQADGKPKCCFFKFSSKIQYNKVVKAQLWIYLRPVKTPTTVFVQILRLIKPMKDGTRYTGIRSLKLDMSPGTGIWQSIDVKTVLQNWLKQPESNLGIEIKALDENGHDLAVTFPGPGEDGLNPFLEVKVTDTPKRSRRDFGLDCDEHSTESRCCRYPLTVDFEAFGWDWIIAPKRYKANYCSGECEFVFLQKYPHTHLVHQANPRGSAGPCCTPTKMSPINMLYFNGKEQIIYGKIPAMVVDRCGCS

SEQ ID NO: 55 - protein, 277 aa, Macaca fascicularis
NENSEQKENVEKEGLCNACTWRQNTKSSRIEAIKIQILSKLRLETAPNISKDAIRQLLPKAPPLRELIDQYDVQRDDSSDGSLEDDDYHATTETIITMPTESDFLMQVDGKPKCCFFKFSSKIQYNKVVKAQLWIYLRPVETPTTVFVQILRLIKPMKDGTRYTGIRSLKLDMNPGTGIWQSIDVKTVLQNWLKQPESNLGIEIKALDENGHDLAVTFPGPGEDGLNPFLEVKVTDTPKRSRRDFGLDCDEHSTESRCCRYPLTVDFEAFGWDWIIA

SEQ ID NO: 56 - protein, 4 aa, Artificial Sequence
  Synthetic Polypeptide
RSRR

SEQ ID NO: 57 - protein, 4 aa, Artificial Sequence
  Synthetic Polypeptide
RVRR

SEQ ID NO: 58 - protein, 5 aa, Artificial Sequence
  Synthetic Polypeptide
CPPCP

SEQ ID NO: 59 - protein, 17 aa, Artificial Sequence
  Synthetic Polypeptide
HYYGMDVWGQGTTVTVS

SEQ ID NO: 60 - protein, 89 aa, Artificial Sequence
  Synthetic Polypeptide
QSVLTQPPSASGTPGQRVTISCSGSSSNIGSNTVNWYQQLPGTAPKLLIYSNNQRPSGVPDRFSGSKSGTSASLAISGLQSEDEADYYC

SEQ ID NO: 61 - protein, 11 aa, Artificial Sequence
  Synthetic Polypeptide
VFGGGTKLTVL

SEQ ID NO: 62 - protein, 33 aa, Artificial Sequence
  Synthetic Polypeptide
PKAPPLRELIDQYDVQRDDSSDGSLEDDDYHAT

SEQ ID NO: 63 - protein, 34 aa, Artificial Sequence
  Synthetic Polypeptide
GLNPFLEVKVTDTPKRSRRDFGLDCDEHSTESRC

SEQ ID NO: 64 - protein, 80 aa, Synthetic Polynucleotide
VDLNENSEQKENVEKEGLCNACTWRQNTKSSRIEAIKIQILSKLRLETAPNISKDVIRQLLPKAPPLRELIDQYDVQRDD

SEQ ID NO: 65 - protein, 418 aa, Synthetic Polynucleotide
MDMRVPAQLLGLLLLWFSGVLGDYKDDDDKHHHHHHLEVLFQGPAEGPAAAAAAAAAAAAAGVGGERSSRPAPSVAPEPDGCPVCVWRQHSRELRLESIKSQILSKLRLKEAPNISREVVKQLLPKAPPLRELIDQYDVQRDDSSDGSLEDDDYHATTETIITMPTESDFLMQVDGKPKCCFFKFSSKIQYNKVVKAQLWIYLRPVETPTTVFVQILRLIKPMKDGTRYTGIRSLKLDMNPGTGIWQSIDVKTVLQNWLKQPESNLGIEIKALDENGHDLAVTFPGPGEDGLNPFLEVKVTDTPKRSRRNLGLDCDEHSSESRCCRYPLTVDFEAFGWDWIIAPKRYKANYCSGQCEYMFMQKYPHTHLVQQANPRGSAGPCCTPTKMSPINMLYFNDKQQIIYGKIPGMVVDRCGCS